European Patent Application EP 4 112 726 A1, published January 4, 2023. Title: MICROORGANISM HAVING INHANCED ACTIVITY OF 3-METHYL-2-OXOBUTANOATE HYDROXYMETHYLTRANSFERASE AND USES THEREOF. Applicant: CJ CheilJedang Corporation. The sequence listing filed with the application follows.

SEQUENCE LISTING (128 sequences)

SEQ ID NO: 1 - DNA, 37 bp, Artificial Sequence
  synthetic_primer
tagatcgaaaggtgcacaaagatgaaaccgaccacca

SEQ ID NO: 2 - DNA, 41 bp, Artificial Sequence
  synthetic_primer
ccgctctagaactagtggatcttaatggaaactgtgttctt

SEQ ID NO: 3 - DNA, 36 bp, Artificial Sequence
  synthetic_primer
tagatcgaaaggtgcacaaagatgaaaccgaccacc

SEQ ID NO: 4 - DNA, 40 bp, Artificial Sequence
  synthetic_primer
ccgctctagaactagtggatcttaatggaaactgtgttct

SEQ ID NO: 5 - DNA, 38 bp, Artificial Sequence
  synthetic_primer
tagatcgaaaggtgcacaaagatgaaaccaaccaccat

SEQ ID NO: 6 - DNA, 41 bp, Artificial Sequence; identical to SEQ ID NO: 2
  synthetic_primer

SEQ ID NO: 7 - DNA, 42 bp, Artificial Sequence
  synthetic_primer
tagatcgaaaggtgcacaaagatgtcattaaagcaaataact

SEQ ID NO: 8 - DNA, 41 bp, Artificial Sequence
  synthetic_primer
ccgctctagaactagtggatcttattggaaactgtgttctt

SEQ ID NO: 9 - DNA, 36 bp, Artificial Sequence
  synthetic_primer
tagatcgaaaggtgcacaaagatgaaacccaccacc

SEQ ID NO: 10 - DNA, 39 bp, Artificial Sequence
  synthetic_primer
ccgctctagaactagtggatcttagttaaatgagtgctc

SEQ ID NO: 11 - DNA, 37 bp, Artificial Sequence; identical to SEQ ID NO: 1
  synthetic_primer

SEQ ID NO: 12 - DNA, 40 bp, Artificial Sequence; identical to SEQ ID NO: 4
  synthetic_primer

SEQ ID NO: 13 - DNA, 36 bp, Artificial Sequence
  synthetic_primer
tagatcgaaaggtgcacaaagatgaaacccaccacg

SEQ ID NO: 14 - DNA, 38 bp, Artificial Sequence
  synthetic_primer
ccgctctagaactagtggatcttactggaaactgtgct

SEQ ID NO: 15 - DNA, 44 bp, Artificial Sequence
  synthetic_primer
tagatcgaaaggtgcacaaagatgaaaactttaaatcatttaaa

SEQ ID NO: 16 - DNA, 39 bp, Artificial Sequence
  synthetic_primer
ccgctctagaactagtggatcttagtcatgttgctctac

SEQ ID NO: 17 - DNA, 37 bp, Artificial Sequence
  synthetic_primer
tagatcgaaaggtgcacaaagatgccagatgtaaccg

SEQ ID NO: 18 - DNA, 36 bp, Artificial Sequence
  synthetic_primer
ccgctctagaactagtggatctcatgcggagaaccc

SEQ ID NO: 19 - DNA, 36 bp, Artificial Sequence
  synthetic_primer
tagatcgaaaggtgcacaaagatgcctgatgtgacc

SEQ ID NO: 20 - DNA, 36 bp, Artificial Sequence
  synthetic_primer
ccgctctagaactagtggatctcatgcggagaatcc

SEQ ID NO: 21 - DNA, 39 bp, Artificial Sequence
  synthetic_primer
tagatcgaaaggtgcacaaagatgtcggtacataaagaa

SEQ ID NO: 22 - DNA, 42 bp, Artificial Sequence
  synthetic_primer
ccgctctagaactagtggatcttaatattgttctttttcgtt

SEQ ID NO: 23 - DNA, 36 bp, Artificial Sequence; identical to SEQ ID NO: 9
  synthetic_primer

SEQ ID NO: 24 - DNA, 40 bp, Artificial Sequence
  synthetic_primer
ccgctctagaactagtggatcttagttgaaagagtgctct

SEQ ID NO: 25 - DNA, 40 bp, Artificial Sequence
  synthetic_primer
tagatcgaaaggtgcacaaagatgtctacagcaaaaaaag

SEQ ID NO: 26 - DNA, 40 bp, Artificial Sequence
  synthetic_primer
ccgctctagaactagtggatcttaatactgttcatcgtca

SEQ ID NO: 27 - DNA, 41 bp, Artificial Sequence
  synthetic_primer
cttgatatcgaattcctgcattcagggtagttgactaaaga

SEQ ID NO: 28 - DNA, 17 bp, Artificial Sequence
  synthetic_primer
ctttgtgcacctttcga

SEQ ID NO: 29 - DNA, 40 bp, Artificial Sequence
  synthetic_primer
tgaattcgagctcggtacccgaaatagcgcttgatgaatc

SEQ ID NO: 30 - DNA, 40 bp, Artificial Sequence
  synthetic_primer
ggttgctacctgcacccggggggcatgagtatagatgtga

SEQ ID NO: 31 - DNA, 40 bp, Artificial Sequence
  synthetic_primer
ctatactcatgccccccgggtgcaggtagcaaccacaaag

SEQ ID NO: 32 - DNA, 40 bp, Artificial Sequence
  synthetic_primer
gtcgactctagaggatcccctatgtggcgttgggtgcagc

SEQ ID NO: 33 - DNA, 40 bp, Artificial Sequence
  synthetic_primer
catctatactcatgccccccttcagggtagttgactaaag

SEQ ID NO: 34 - DNA, 40 bp, Artificial Sequence
  synthetic_primer
tgtggttgctacctgcacccttaatggaaactgtgttctt

SEQ ID NO: 35 - DNA, 20 bp, Artificial Sequence
  synthetic_primer
cccacccggtgtcattcgac

SEQ ID NO: 36 - DNA, 19 bp, Artificial Sequence
  synthetic_primer
gcgcatccagctcatcggt

SEQ ID NO: 37 - protein, 264 aa, Artificial Sequence
  synthetic_PanB WT
MKPTTISLLQKYKQEKKRFATITAYDYSFAKLFADEGLNVMLVGDSLGMTVQGHDSTLPVTVADIAYHTAAVRRGAPNCLLLADLPFMAYATPEQAFENAATVMRAGANMVKIEGGEWLVETVQMLTERAVPVCGHLGLTPQSVNIFGGYKVQGRGDEAGDQLLSDALALEAAGAQLLVLECVPVELAKRITEALAIPVIGIGAGNVTDGQILVMHDAFGITGGHIPKFAKNFLAETGDIRAAVRQYMAEVESGVYPGEEHSFH

SEQ ID NO: 38 - DNA, 40 bp, Artificial Sequence
  synthetic_primer
gtttctaccagccactcggagccttcaattttgaccatgt

SEQ ID NO: 39 - DNA, 40 bp, Artificial Sequence
  synthetic_primer
acatggtcaaaattgaaggctccgagtggctggtagaaac

SEQ ID NO: 40 - DNA, 40 bp, Artificial Sequence
  synthetic_primer
gtttctaccagccactcgcagccttcaattttgaccatgt

SEQ ID NO: 41 - DNA, 40 bp, Artificial Sequence
  synthetic_primer
acatggtcaaaattgaaggctgcgagtggctggtagaaac

SEQ ID NO: 42 - DNA, 40 bp, Artificial Sequence
  synthetic_primer
gtttctaccagccactccaggccttcaattttgaccatgt

SEQ ID NO: 43 - DNA, 40 bp, Artificial Sequence
  synthetic_primer
acatggtcaaaattgaaggcctggagtggctggtagaaac

SEQ ID NO: 44 - DNA, 40 bp, Artificial Sequence
  synthetic_primer
gtttctaccagccactcgatgccttcaattttgaccatgt

SEQ ID NO: 45 - DNA, 40 bp, Artificial Sequence
  synthetic_primer
acatggtcaaaattgaaggcatcgagtggctggtagaaac

SEQ ID NO: 46 - DNA, 40 bp, Artificial Sequence
  synthetic_primer
gtttctaccagccactcggtgccttcaattttgaccatgt

SEQ ID NO: 47 - DNA, 40 bp, Artificial Sequence
  synthetic_primer
acatggtcaaaattgaaggcaccgagtggctggtagaaac

SEQ ID NO: 48 - DNA, 40 bp, Artificial Sequence
  synthetic_primer
gtttctaccagccactccacgccttcaattttgaccatgt

SEQ ID NO: 49 - DNA, 40 bp, Artificial Sequence
  synthetic_primer
acatggtcaaaattgaaggcgtggagtggctggtagaaac

SEQ ID NO: 50 - DNA, 40 bp, Artificial Sequence
  synthetic_primer
gtttctaccagccactccatgccttcaattttgaccatgt

SEQ ID NO: 51 - DNA, 40 bp, Artificial Sequence
  synthetic_primer
acatggtcaaaattgaaggcatggagtggctggtagaaac

SEQ ID NO: 52 - DNA, 40 bp, Artificial Sequence
  synthetic_primer
gtttctaccagccactcatcgccttcaattttgaccatgt

SEQ ID NO: 53 - DNA, 40 bp, Artificial Sequence
  synthetic_primer
acatggtcaaaattgaaggcgatgagtggctggtagaaac

SEQ ID NO: 54 - DNA, 40 bp, Artificial Sequence
  synthetic_primer
gtttctaccagccactcttcgccttcaattttgaccatgt

SEQ ID NO: 55 - DNA, 40 bp, Artificial Sequence
  synthetic_primer
acatggtcaaaattgaaggcgaagagtggctggtagaaac

SEQ ID NO: 56 - DNA, 40 bp, Artificial Sequence
  synthetic_primer
gtttctaccagccactcgttgccttcaattttgaccatgt

SEQ ID NO: 57 - DNA, 40 bp, Artificial Sequence
  synthetic_primer
acatggtcaaaattgaaggcaacgagtggctggtagaaac

SEQ ID NO: 58 - DNA, 40 bp, Artificial Sequence
  synthetic_primer
gtttctaccagccactcctggccttcaattttgaccatgt

SEQ ID NO: 59 - DNA, 40 bp, Artificial Sequence
  synthetic_primer
acatggtcaaaattgaaggccaggagtggctggtagaaac

SEQ ID NO: 60 - DNA, 40 bp, Artificial Sequence
  synthetic_primer
gtttctaccagccactctgcgccttcaattttgaccatgt

SEQ ID NO: 61 - DNA, 40 bp, Artificial Sequence
  synthetic_primer
acatggtcaaaattgaaggcgcagagtggctggtagaaac

SEQ ID NO: 62 - protein, 264 aa, Artificial Sequence
  synthetic_PanB with G116A mutation
MKPTTISLLQKYKQEKKRFATITAYDYSFAKLFADEGLNVMLVGDSLGMTVQGHDSTLPVTVADIAYHTAAVRRGAPNCLLLADLPFMAYATPEQAFENAATVMRAGANMVKIEGAEWLVETVQMLTERAVPVCGHLGLTPQSVNIFGGYKVQGRGDEAGDQLLSDALALEAAGAQLLVLECVPVELAKRITEALAIPVIGIGAGNVTDGQILVMHDAFGITGGHIPKFAKNFLAETGDIRAAVRQYMAEVESGVYPGEEHSFH

SEQ ID NO: 63 - protein, 264 aa, Artificial Sequence
  synthetic_PanB with G116N mutation
MKPTTISLLQKYKQEKKRFATITAYDYSFAKLFADEGLNVMLVGDSLGMTVQGHDSTLPVTVADIAYHTAAVRRGAPNCLLLADLPFMAYATPEQAFENAATVMRAGANMVKIEGNEWLVETVQMLTERAVPVCGHLGLTPQSVNIFGGYKVQGRGDEAGDQLLSDALALEAAGAQLLVLECVPVELAKRITEALAIPVIGIGAGNVTDGQILVMHDAFGITGGHIPKFAKNFLAETGDIRAAVRQYMAEVESGVYPGEEHSFH

SEQ ID NO: 64 - protein, 264 aa, Artificial Sequence
  synthetic_PanB with G116T mutation
MKPTTISLLQKYKQEKKRFATITAYDYSFAKLFADEGLNVMLVGDSLGMTVQGHDSTLPVTVADIAYHTAAVRRGAPNCLLLADLPFMAYATPEQAFENAATVMRAGANMVKIEGTEWLVETVQMLTERAVPVCGHLGLTPQSVNIFGGYKVQGRGDEAGDQLLSDALALEAAGAQLLVLECVPVELAKRITEALAIPVIGIGAGNVTDGQILVMHDAFGITGGHIPKFAKNFLAETGDIRAAVRQYMAEVESGVYPGEEHSFH

SEQ ID NO: 65 - protein, 264 aa, Artificial Sequence
  synthetic_PanB with G116E mutation
MKPTTISLLQKYKQEKKRFATITAYDYSFAKLFADEGLNVMLVGDSLGMTVQGHDSTLPVTVADIAYHTAAVRRGAPNCLLLADLPFMAYATPEQAFENAATVMRAGANMVKIEGEEWLVETVQMLTERAVPVCGHLGLTPQSVNIFGGYKVQGRGDEAGDQLLSDALALEAAGAQLLVLECVPVELAKRITEALAIPVIGIGAGNVTDGQILVMHDAFGITGGHIPKFAKNFLAETGDIRAAVRQYMAEVESGVYPGEEHSFH

SEQ ID NO: 66 - protein, 264 aa, Artificial Sequence
  synthetic_PanB with G116S mutation
MKPTTISLLQKYKQEKKRFATITAYDYSFAKLFADEGLNVMLVGDSLGMTVQGHDSTLPVTVADIAYHTAAVRRGAPNCLLLADLPFMAYATPEQAFENAATVMRAGANMVKIEGSEWLVETVQMLTERAVPVCGHLGLTPQSVNIFGGYKVQGRGDEAGDQLLSDALALEAAGAQLLVLECVPVELAKRITEALAIPVIGIGAGNVTDGQILVMHDAFGITGGHIPKFAKNFLAETGDIRAAVRQYMAEVESGVYPGEEHSFH

SEQ ID NO: 67 - protein, 264 aa, Artificial Sequence
  synthetic_PanB with G116V mutation
MKPTTISLLQKYKQEKKRFATITAYDYSFAKLFADEGLNVMLVGDSLGMTVQGHDSTLPVTVADIAYHTAAVRRGAPNCLLLADLPFMAYATPEQAFENAATVMRAGANMVKIEGVEWLVETVQMLTERAVPVCGHLGLTPQSVNIFGGYKVQGRGDEAGDQLLSDALALEAAGAQLLVLECVPVELAKRITEALAIPVIGIGAGNVTDGQILVMHDAFGITGGHIPKFAKNFLAETGDIRAAVRQYMAEVESGVYPGEEHSFH

SEQ ID NO: 68 - protein, 264 aa, Artificial Sequence
  synthetic_PanB with G116I mutation
MKPTTISLLQKYKQEKKRFATITAYDYSFAKLFADEGLNVMLVGDSLGMTVQGHDSTLPVTVADIAYHTAAVRRGAPNCLLLADLPFMAYATPEQAFENAATVMRAGANMVKIEGIEWLVETVQMLTERAVPVCGHLGLTPQSVNIFGGYKVQGRGDEAGDQLLSDALALEAAGAQLLVLECVPVELAKRITEALAIPVIGIGAGNVTDGQILVMHDAFGITGGHIPKFAKNFLAETGDIRAAVRQYMAEVESGVYPGEEHSFH

SEQ ID NO: 69 - protein, 264 aa, Artificial Sequence
  synthetic_PanB with G116L mutation
MKPTTISLLQKYKQEKKRFATITAYDYSFAKLFADEGLNVMLVGDSLGMTVQGHDSTLPVTVADIAYHTAAVRRGAPNCLLLADLPFMAYATPEQAFENAATVMRAGANMVKIEGLEWLVETVQMLTERAVPVCGHLGLTPQSVNIFGGYKVQGRGDEAGDQLLSDALALEAAGAQLLVLECVPVELAKRITEALAIPVIGIGAGNVTDGQILVMHDAFGITGGHIPKFAKNFLAETGDIRAAVRQYMAEVESGVYPGEEHSFH

SEQ ID NO: 70 - protein, 264 aa, Artificial Sequence
  synthetic_PanB with G116D mutation
MKPTTISLLQKYKQEKKRFATITAYDYSFAKLFADEGLNVMLVGDSLGMTVQGHDSTLPVTVADIAYHTAAVRRGAPNCLLLADLPFMAYATPEQAFENAATVMRAGANMVKIEGDEWLVETVQMLTERAVPVCGHLGLTPQSVNIFGGYKVQGRGDEAGDQLLSDALALEAAGAQLLVLECVPVELAKRITEALAIPVIGIGAGNVTDGQILVMHDAFGITGGHIPKFAKNFLAETGDIRAAVRQYMAEVESGVYPGEEHSFH

SEQ ID NO: 71 - protein, 264 aa, Artificial Sequence
  synthetic_PanB with G116C mutation
MKPTTISLLQKYKQEKKRFATITAYDYSFAKLFADEGLNVMLVGDSLGMTVQGHDSTLPVTVADIAYHTAAVRRGAPNCLLLADLPFMAYATPEQAFENAATVMRAGANMVKIEGCEWLVETVQMLTERAVPVCGHLGLTPQSVNIFGGYKVQGRGDEAGDQLLSDALALEAAGAQLLVLECVPVELAKRITEALAIPVIGIGAGNVTDGQILVMHDAFGITGGHIPKFAKNFLAETGDIRAAVRQYMAEVESGVYPGEEHSFH

SEQ ID NO: 72 - protein, 264 aa, Artificial Sequence
  synthetic_PanB with G116Q mutation
MKPTTISLLQKYKQEKKRFATITAYDYSFAKLFADEGLNVMLVGDSLGMTVQGHDSTLPVTVADIAYHTAAVRRGAPNCLLLADLPFMAYATPEQAFENAATVMRAGANMVKIEGQEWLVETVQMLTERAVPVCGHLGLTPQSVNIFGGYKVQGRGDEAGDQLLSDALALEAAGAQLLVLECVPVELAKRITEALAIPVIGIGAGNVTDGQILVMHDAFGITGGHIPKFAKNFLAETGDIRAAVRQYMAEVESGVYPGEEHSFH

SEQ ID NO: 73 - protein, 264 aa, Artificial Sequence
  synthetic_PanB with G116M mutation
MKPTTISLLQKYKQEKKRFATITAYDYSFAKLFADEGLNVMLVGDSLGMTVQGHDSTLPVTVADIAYHTAAVRRGAPNCLLLADLPFMAYATPEQAFENAATVMRAGANMVKIEGMEWLVETVQMLTERAVPVCGHLGLTPQSVNIFGGYKVQGRGDEAGDQLLSDALALEAAGAQLLVLECVPVELAKRITEALAIPVIGIGAGNVTDGQILVMHDAFGITGGHIPKFAKNFLAETGDIRAAVRQYMAEVESGVYPGEEHSFH

SEQ ID NO: 74 - DNA, 40 bp, Artificial Sequence
  primer
agatcgaaaggtgcacaaagatgaaaccgaccaccatctc

SEQ ID NO: 75 - DNA, 40 bp, Artificial Sequence
  primer
aggggcgcggcgatgaacgcggcgatcaactgctcagcga

SEQ ID NO: 76 - DNA, 40 bp, Artificial Sequence
  primer
ctgagcagttgatcgccgcgttcatcgccgcgcccctgaa

SEQ ID NO: 77 - DNA, 40 bp, Artificial Sequence
  primer
cgctctagaactagtggatcttaatggaaactgtgttctt

SEQ ID NO: 78 - DNA, 40 bp, Artificial Sequence
  primer
aggggcgcggcgatgaatccggcgatcaactgctcagcga

SEQ ID NO: 79 - DNA, 40 bp, Artificial Sequence
  primer
ctgagcagttgatcgccggattcatcgccgcgcccctgaa

SEQ ID NO: 80 - DNA, 40 bp, Artificial Sequence
  primer
aggggcgcggcgatgaatacggcgatcaactgctcagcga

SEQ ID NO: 81 - DNA, 40 bp, Artificial Sequence
  primer
ctgagcagttgatcgccgtattcatcgccgcgcccctgaa

SEQ ID NO: 82 - DNA, 40 bp, Artificial Sequence
  primer
aggggcgcggcgatgaatgcggcgatcaactgctcagcga

SEQ ID NO: 83 - DNA, 40 bp, Artificial Sequence
  primer
ctgagcagttgatcgccgcattcatcgccgcgcccctgaa

SEQ ID NO: 84 - DNA, 40 bp, Artificial Sequence
  primer
aggggcgcggcgatgaaccaggcgatcaactgctcagcga

SEQ ID NO: 85 - DNA, 40 bp, Artificial Sequence
  primer
ctgagcagttgatcgcctggttcatcgccgcgcccctgaa

SEQ ID NO: 86 - DNA, 40 bp, Artificial Sequence
  primer
aggggcgcggcgatgaacacggcgatcaactgctcagcga

SEQ ID NO: 87 - DNA, 40 bp, Artificial Sequence
  primer
ctgagcagttgatcgccgtgttcatcgccgcgcccctgaa

SEQ ID NO: 88 - DNA, 40 bp, Artificial Sequence
  primer
aggggcgcggcgatgaactgggcgatcaactgctcagcga

SEQ ID NO: 89 - DNA, 40 bp, Artificial Sequence
  primer
ctgagcagttgatcgcccagttcatcgccgcgcccctgaa

SEQ ID NO: 90 - DNA, 40 bp, Artificial Sequence
  primer
aggggcgcggcgatgaaatcggcgatcaactgctcagcga

SEQ ID NO: 91 - DNA, 40 bp, Artificial Sequence
  primer
ctgagcagttgatcgccgatttcatcgccgcgcccctgaa

SEQ ID NO: 92 - DNA, 40 bp, Artificial Sequence
  primer
aggggcgcggcgatgaaaccggcgatcaactgctcagcga

SEQ ID NO: 93 - DNA, 40 bp, Artificial Sequence
  primer
ctgagcagttgatcgccggtttcatcgccgcgcccctgaa

SEQ ID NO: 94 - DNA, 40 bp, Artificial Sequence
  primer
aggggcgcggcgatgaaaagggcgatcaactgctcagcga

SEQ ID NO: 95 - DNA, 40 bp, Artificial Sequence
  primer
ctgagcagttgatcgcccttttcatcgccgcgcccctgaa

SEQ ID NO: 96 - DNA, 40 bp, Artificial Sequence
  primer
aggggcgcggcgatgaagtgggcgatcaactgctcagcga

SEQ ID NO: 97 - DNA, 40 bp, Artificial Sequence
  primer
ctgagcagttgatcgcccacttcatcgccgcgcccctgaa

SEQ ID NO: 98 - DNA, 40 bp, Artificial Sequence
  primer
aggggcgcggcgatgaaatgggcgatcaactgctcagcga

SEQ ID NO: 99 - DNA, 40 bp, Artificial Sequence
  primer
ctgagcagttgatcgcccatttcatcgccgcgcccctgaa

SEQ ID NO: 100 - DNA, 40 bp, Artificial Sequence
  primer
aggggcgcggcgatgaagatggcgatcaactgctcagcga

SEQ ID NO: 101 - DNA, 40 bp, Artificial Sequence
  primer
ctgagcagttgatcgccatcttcatcgccgcgcccctgaa

SEQ ID NO: 102 - DNA, 40 bp, Artificial Sequence
  primer
aggggcgcggcgatgaacagggcgatcaactgctcagcga

SEQ ID NO: 103 - DNA, 40 bp, Artificial Sequence
  primer
ctgagcagttgatcgccctgttcatcgccgcgcccctgaa

SEQ ID NO: 104 - DNA, 40 bp, Artificial Sequence
  primer
aggggcgcggcgatgaaaacggcgatcaactgctcagcga

SEQ ID NO: 105 - DNA, 40 bp, Artificial Sequence
  primer
ctgagcagttgatcgccgttttcatcgccgcgcccctgaa

SEQ ID NO: 106 - DNA, 40 bp, Artificial Sequence; identical to SEQ ID NO: 102
  primer

SEQ ID NO: 107 - DNA, 40 bp, Artificial Sequence; identical to SEQ ID NO: 103
  primer

SEQ ID NO: 108 - DNA, 40 bp, Artificial Sequence
  primer
cttgatatcgaattcctgcattcagggtagttgactaaag

SEQ ID NO: 109 - DNA, 40 bp, Artificial Sequence
  primer
gagatggtggtcggtttcatctttgtgcacctttcgatct

SEQ ID NO: 110 - protein, 264 aa, Artificial Sequence
  PanB with A159L mutation
MKPTTISLLQKYKQEKKRFATITAYDYSFAKLFADEGLNVMLVGDSLGMTVQGHDSTLPVTVADIAYHTAAVRRGAPNCLLLADLPFMAYATPEQAFENAATVMRAGANMVKIEGGEWLVETVQMLTERAVPVCGHLGLTPQSVNIFGGYKVQGRGDELGDQLLSDALALEAAGAQLLVLECVPVELAKRITEALAIPVIGIGAGNVTDGQILVMHDAFGITGGHIPKFAKNFLAETGDIRAAVRQYMAEVESGVYPGEEHSFH

SEQ ID NO: 111 - protein, 264 aa, Artificial Sequence
  PanB with A159R mutation
MKPTTISLLQKYKQEKKRFATITAYDYSFAKLFADEGLNVMLVGDSLGMTVQGHDSTLPVTVADIAYHTAAVRRGAPNCLLLADLPFMAYATPEQAFENAATVMRAGANMVKIEGGEWLVETVQMLTERAVPVCGHLGLTPQSVNIFGGYKVQGRGDERGDQLLSDALALEAAGAQLLVLECVPVELAKRITEALAIPVIGIGAGNVTDGQILVMHDAFGITGGHIPKFAKNFLAETGDIRAAVRQYMAEVESGVYPGEEHSFH

SEQ ID NO: 112 - protein, 264 aa, Artificial Sequence
  PanB with A159S mutation
MKPTTISLLQKYKQEKKRFATITAYDYSFAKLFADEGLNVMLVGDSLGMTVQGHDSTLPVTVADIAYHTAAVRRGAPNCLLLADLPFMAYATPEQAFENAATVMRAGANMVKIEGGEWLVETVQMLTERAVPVCGHLGLTPQSVNIFGGYKVQGRGDESGDQLLSDALALEAAGAQLLVLECVPVELAKRITEALAIPVIGIGAGNVTDGQILVMHDAFGITGGHIPKFAKNFLAETGDIRAAVRQYMAEVESGVYPGEEHSFH

SEQ ID NO: 113 - protein, 264 aa, Artificial Sequence
  PanB with A159Y mutation
MKPTTISLLQKYKQEKKRFATITAYDYSFAKLFADEGLNVMLVGDSLGMTVQGHDSTLPVTVADIAYHTAAVRRGAPNCLLLADLPFMAYATPEQAFENAATVMRAGANMVKIEGGEWLVETVQMLTERAVPVCGHLGLTPQSVNIFGGYKVQGRGDEYGDQLLSDALALEAAGAQLLVLECVPVELAKRITEALAIPVIGIGAGNVTDGQILVMHDAFGITGGHIPKFAKNFLAETGDIRAAVRQYMAEVESGVYPGEEHSFH

SEQ ID NO: 114 - protein, 264 aa, Artificial Sequence
  PanB with A159C mutation
MKPTTISLLQKYKQEKKRFATITAYDYSFAKLFADEGLNVMLVGDSLGMTVQGHDSTLPVTVADIAYHTAAVRRGAPNCLLLADLPFMAYATPEQAFENAATVMRAGANMVKIEGGEWLVETVQMLTERAVPVCGHLGLTPQSVNIFGGYKVQGRGDECGDQLLSDALALEAAGAQLLVLECVPVELAKRITEALAIPVIGIGAGNVTDGQILVMHDAFGITGGHIPKFAKNFLAETGDIRAAVRQYMAEVESGVYPGEEHSFH

SEQ ID NO: 115 - protein, 264 aa, Artificial Sequence
  PanB with A159P mutation
MKPTTISLLQKYKQEKKRFATITAYDYSFAKLFADEGLNVMLVGDSLGMTVQGHDSTLPVTVADIAYHTAAVRRGAPNCLLLADLPFMAYATPEQAFENAATVMRAGANMVKIEGGEWLVETVQMLTERAVPVCGHLGLTPQSVNIFGGYKVQGRGDEPGDQLLSDALALEAAGAQLLVLECVPVELAKRITEALAIPVIGIGAGNVTDGQILVMHDAFGITGGHIPKFAKNFLAETGDIRAAVRQYMAEVESGVYPGEEHSFH

SEQ ID NO: 116 - protein, 264 aa, Artificial Sequence
  PanB with A159H mutation
MKPTTISLLQKYKQEKKRFATITAYDYSFAKLFADEGLNVMLVGDSLGMTVQGHDSTLPVTVADIAYHTAAVRRGAPNCLLLADLPFMAYATPEQAFENAATVMRAGANMVKIEGGEWLVETVQMLTERAVPVCGHLGLTPQSVNIFGGYKVQGRGDEHGDQLLSDALALEAAGAQLLVLECVPVELAKRITEALAIPVIGIGAGNVTDGQILVMHDAFGITGGHIPKFAKNFLAETGDIRAAVRQYMAEVESGVYPGEEHSFH

SEQ ID NO: 117 - protein, 264 aa, Artificial Sequence
  PanB with A159I mutation
MKPTTISLLQKYKQEKKRFATITAYDYSFAKLFADEGLNVMLVGDSLGMTVQGHDSTLPVTVADIAYHTAAVRRGAPNCLLLADLPFMAYATPEQAFENAATVMRAGANMVKIEGGEWLVETVQMLTERAVPVCGHLGLTPQSVNIFGGYKVQGRGDEIGDQLLSDALALEAAGAQLLVLECVPVELAKRITEALAIPVIGIGAGNVTDGQILVMHDAFGITGGHIPKFAKNFLAETGDIRAAVRQYMAEVESGVYPGEEHSFH

SEQ ID NO: 118 - protein, 264 aa, Artificial Sequence
  PanB with A159T mutation
MKPTTISLLQKYKQEKKRFATITAYDYSFAKLFADEGLNVMLVGDSLGMTVQGHDSTLPVTVADIAYHTAAVRRGAPNCLLLADLPFMAYATPEQAFENAATVMRAGANMVKIEGGEWLVETVQMLTERAVPVCGHLGLTPQSVNIFGGYKVQGRGDETGDQLLSDALALEAAGAQLLVLECVPVELAKRITEALAIPVIGIGAGNVTDGQILVMHDAFGITGGHIPKFAKNFLAETGDIRAAVRQYMAEVESGVYPGEEHSFH

SEQ ID NO: 119 - protein, 264 aa, Artificial Sequence
  PanB with A159K mutation
MKPTTISLLQKYKQEKKRFATITAYDYSFAKLFADEGLNVMLVGDSLGMTVQGHDSTLPVTVADIAYHTAAVRRGAPNCLLLADLPFMAYATPEQAFENAATVMRAGANMVKIEGGEWLVETVQMLTERAVPVCGHLGLTPQSVNIFGGYKVQGRGDEKGDQLLSDALALEAAGAQLLVLECVPVELAKRITEALAIPVIGIGAGNVTDGQILVMHDAFGITGGHIPKFAKNFLAETGDIRAAVRQYMAEVESGVYPGEEHSFH

SEQ ID NO: 120 - protein, 264 aa, Artificial Sequence
  PanB with A159V mutation
MKPTTISLLQKYKQEKKRFATITAYDYSFAKLFADEGLNVMLVGDSLGMTVQGHDSTLPVTVADIAYHTAAVRRGAPNCLLLADLPFMAYATPEQAFENAATVMRAGANMVKIEGGEWLVETVQMLTERAVPVCGHLGLTPQSVNIFGGYKVQGRGDEVGDQLLSDALALEAAGAQLLVLECVPVELAKRITEALAIPVIGIGAGNVTDGQILVMHDAFGITGGHIPKFAKNFLAETGDIRAAVRQYMAEVESGVYPGEEHSFH

SEQ ID NO: 121 - protein, 264 aa, Artificial Sequence
  PanB with A159M mutation
MKPTTISLLQKYKQEKKRFATITAYDYSFAKLFADEGLNVMLVGDSLGMTVQGHDSTLPVTVADIAYHTAAVRRGAPNCLLLADLPFMAYATPEQAFENAATVMRAGANMVKIEGGEWLVETVQMLTERAVPVCGHLGLTPQSVNIFGGYKVQGRGDEMGDQLLSDALALEAAGAQLLVLECVPVELAKRITEALAIPVIGIGAGNVTDGQILVMHDAFGITGGHIPKFAKNFLAETGDIRAAVRQYMAEVESGVYPGEEHSFH

SEQ ID NO: 122 - protein, 264 aa, Artificial Sequence
  PanB with A159D mutation
MKPTTISLLQKYKQEKKRFATITAYDYSFAKLFADEGLNVMLVGDSLGMTVQGHDSTLPVTVADIAYHTAAVRRGAPNCLLLADLPFMAYATPEQAFENAATVMRAGANMVKIEGGEWLVETVQMLTERAVPVCGHLGLTPQSVNIFGGYKVQGRGDEDGDQLLSDALALEAAGAQLLVLECVPVELAKRITEALAIPVIGIGAGNVTDGQILVMHDAFGITGGHIPKFAKNFLAETGDIRAAVRQYMAEVESGVYPGEEHSFH

SEQ ID NO: 123 - protein, 264 aa, Artificial Sequence
  PanB with A159E mutation
MKPTTISLLQKYKQEKKRFATITAYDYSFAKLFADEGLNVMLVGDSLGMTVQGHDSTLPVTVADIAYHTAAVRRGAPNCLLLADLPFMAYATPEQAFENAATVMRAGANMVKIEGGEWLVETVQMLTERAVPVCGHLGLTPQSVNIFGGYKVQGRGDEEGDQLLSDALALEAAGAQLLVLECVPVELAKRITEALAIPVIGIGAGNVTDGQILVMHDAFGITGGHIPKFAKNFLAETGDIRAAVRQYMAEVESGVYPGEEHSFH

SEQ ID NO: 124 - protein, 264 aa, Artificial Sequence
  PanB with A159N mutation
MKPTTISLLQKYKQEKKRFATITAYDYSFAKLFADEGLNVMLVGDSLGMTVQGHDSTLPVTVADIAYHTAAVRRGAPNCLLLADLPFMAYATPEQAFENAATVMRAGANMVKIEGGEWLVETVQMLTERAVPVCGHLGLTPQSVNIFGGYKVQGRGDENGDQLLSDALALEAAGAQLLVLECVPVELAKRITEALAIPVIGIGAGNVTDGQILVMHDAFGITGGHIPKFAKNFLAETGDIRAAVRQYMAEVESGVYPGEEHSFH

SEQ ID NO: 125 - protein, 264 aa, Artificial Sequence
  PanB with A159Q mutation
MKPTTISLLQKYKQEKKRFATITAYDYSFAKLFADEGLNVMLVGDSLGMTVQGHDSTLPVTVADIAYHTAAVRRGAPNCLLLADLPFMAYATPEQAFENAATVMRAGANMVKIEGGEWLVETVQMLTERAVPVCGHLGLTPQSVNIFGGYKVQGRGDEQGDQLLSDALALEAAGAQLLVLECVPVELAKRITEALAIPVIGIGAGNVTDGQILVMHDAFGITGGHIPKFAKNFLAETGDIRAAVRQYMAEVESGVYPGEEHSFH

SEQ ID NO: 126 - DNA, 40 bp, Artificial Sequence
  primer
gtttctaccagccactcggcgccttcaattttgaccatgt

SEQ ID NO: 127 - DNA, 40 bp, Artificial Sequence
  primer
tggtcaaaattgaaggcgccgagtggctggtagaaaccgt

SEQ ID NO: 128 - protein, 264 aa, Artificial Sequence
  PanB with G116A and A159L mutation
MKPTTISLLQKYKQEKKRFATITAYDYSFAKLFADEGLNVMLVGDSLGMTVQGHDSTLPVTVADIAYHTAAVRRGAPNCLLLADLPFMAYATPEQAFENAATVMRAGANMVKIEGAEWLVETVQMLTERAVPVCGHLGLTPQSVNIFGGYKVQGRGDELGDQLLSDALALEAAGAQLLVLECVPVELAKRITEALAIPVIGIGAGNVTDGQILVMHDAFGITGGHIPKFAKNFLAETGDIRAAVRQYMAEVESGVYPGEEHSFH